European Patent Application EP 4 299 589 A1, published January 3, 2024. Title: ANTI-HUMAN CD73 ANTIBODY AND USE THEREOF. Applicant: NOVOPROTEIN SCIENTIFIC INC.; NOVOPROTEIN SCIENTIFIC (SHANGHAI) INC. The sequence listing filed with the application follows.

SEQUENCE LISTING (47 sequences)

SEQ ID NO: 1 - protein, 108 aa, Artificial Sequence
  CQ137VL
DILMTQSPSSMYASLGERVTITCKASQDINTYLTWFQQKPGKSPKTLIYRANILVDGVPSRFSGSGSGQDYSLTISSLEFEDMGIYYCLQYDEFPLTFGAGTKLELKR

SEQ ID NO: 2 - protein, 117 aa, Artificial Sequence
  CQ137VH
EVQLQQSGPELVKPGASVKISCKASGYSFTGYYIHWVKQSHVKSLEWIGRINPYNGATTYNQNFKDKASLTVDKSSSTAYMELHSLTSEDSAVYYCARFHYGAPDYWGQGTTLTVSS

SEQ ID NO: 3 - protein, 330 aa, Artificial Sequence [sequence omitted]

SEQ ID NO: 4 - protein, 106 aa, Artificial Sequence
  CQ137-CL
TVAAPSVFIFPPSDEQLKSGTASVVCLLNNFYPREAKVQWKVDNALQSGNSQESVTEQDSKDSTYSLSSTLTLSKADYEKHKVYACEVTHQGLSSPVTKSFNRGEC

SEQ ID NO: 5 - protein, 117 aa, Artificial Sequence
  hCQ137-1VH
QVQLVQSGAEVKKPGASVKVSCKASGYTFTGYYIHWVRQAPGQGLEWMGRINPYNGATTYNQNFKDRVTMTVDKSTSTAYMELRSLRSDDTAVYYCARFHYGAPDYWGQGTLVTVSS

SEQ ID NO: 6 - protein, 108 aa, Artificial Sequence
  hCQ137-1VL
DIQMTQSPSSLSASVGDRVTITCKASQDINTYLTWFQQKPGKAPKTLIYRANILVDGVPSRFSGSGSGQDYTLTISSLQPEDFATYYCLQYDEFPLTFGGGTKVEIKR

SEQ ID NO: 7 - protein, 117 aa, Artificial Sequence
  hCQ137-2VH
QVQLVQSGAEVKKPGASVKVSCKASGYSFTGYYIHWVRQAPGQGLEWMGRINPYNGATTYNQNFKDRVTMTVDKSTSTAYMELRSLRSDDTAVYYCARFHYGAPDYWGQGTLVTVSS

SEQ ID NO: 8 - protein, 108 aa, Artificial Sequence
  hCQ137-2VL
DIQMTQSPSSLSASVGDRVTITCKASQDINTYLTWFQQKPGKAPKSLIYRANILVDGVPSRFSGSGSGTDFTLTISSLQPEDFATYYCLQYDEFPLTFGGGTKVEIKR

SEQ ID NO: 9 - protein, 117 aa, Artificial Sequence
  hCQ137-3VH
QVQLVQSGAEVKKPGSSVKVSCKASGYSFTGYYIHWVRQAPGQGLEWMGRINPYNGATTYNQNFKDRVTITVDKSTSTAYMELSSLRSEDTAVYYCARFHYGAPDYWGQGTLVTVSS

SEQ ID NO: 10 - protein, 108 aa, Artificial Sequence
  hCQ137-3VL
DIQMTQSPSSLSASVGDRVTITCKASQDINTYLTWYQQKPGKAPKTLIYRANILVDGVPSRFSGSGSGTDFTLTISSLQPEDFATYYCLQYDEFPLTFGGGTKVEIKR

SEQ ID NO: 11 - DNA, 351 bp, Artificial Sequence
  CQ137VH
gaggttcagctgcagcagtctggacctgagctggtgaagcctggggcttcagtgaagatatcctgcaaggcttctggttactcattcactggctactacatccactgggtgaagcaaagccatgtaaagagccttgagtggattggacgtattaatccttacaatggtgctactacctacaaccagaatttcaaggacaaggccagcttgactgtagataagtcctccagcacagcctacatggagctccacagcctgacatctgaggactctgcagtctattactgtgcaagattccactacggtgcccctgactactggggccaaggcaccactctcacagtctcctcg

SEQ ID NO: 12 - DNA, 324 bp, Artificial Sequence
  CQ137VL
gatattctgatgacccaatctccatcttccatgtatgcatctctaggagagagagtcactatcacttgcaaggcgagtcaggacattaatacctatttaacttggttccagcagaaaccagggaaatctcctaagaccctgatctatcgtgcaaacatattggtagatggggtcccatcaaggttcagtggcagtggatctgggcaagattattctctcaccatcagcagcctggagtttgaagatatgggaatttattattgtctacagtatgatgagtttccgctcacgttcggtgctgggaccaagctggagctgaaacgt

SEQ ID NO: 13 - DNA, 993 bp, Artificial Sequence
  CQ137-CH
gcctccaccaagggcccatcggtcttccccctggcaccctcctccaagagcacctctgggggcacagcggccctgggctgcctggtcaaggactacttccccgaaccggtgacggtgtcgtggaactcaggcgccctgaccagcggcgtgcacaccttcccggctgtcctacagtcctcaggactctactccctcagcagcgtggtgaccgtgccctccagcagcttgggcacccagacctacatctgcaacgtgaatcacaagcccagcaacaccaaggtggacaagaaagttgagcccaaatcttgtgacaaaactcacacatgcccaccgtgcccagcacctgaactcctggggggaccgtcagtcttcctcttccccccaaaacccaaggacaccctcatgatctcccggacccctgaggtcacatgcgtggtggtggacgtgagccacgaagaccctgaggtcaagttcaactggtacgtggacggcgtggaggtgcataatgccaagacaaagccgcgggaggagcagtacaacagcacgtaccgggtggtcagcgtcctcaccgtcctgcaccaggactggctgaatggcaaggagtacaagtgcaaggtctccaacaaagccctcccagcccccatcgagaaaaccatctccaaagccaaagggcagccccgagaaccacaggtgtacaccctgcccccatcccgggatgagctgaccaagaaccaggtcagcctgacctgcctggtcaaaggcttctatcccagcgacatcgccgtggagtgggagagcaatgggcagccggagaacaactacaagaccacgcctcccgtgctggactccgacggctccttcttcctctacagcaagctcaccgtggacaagagcaggtggcagcaggggaacgtcttctcatgctccgtgatgcatgaggctctgcacaaccactacacgcagaagagcctctccctgtctccgggtaaatga

SEQ ID NO: 14 - DNA, 321 bp, Artificial Sequence
  CQ137-CL
acggtggctgcaccatctgtcttcatcttcccgccatctgatgagcagttgaaatctggaactgcctctgttgtgtgcctgctgaataacttctatcccagagaggccaaagtacagtggaaggtggataacgccctccaatcgggtaactcccaggagagtgtcacagagcaggacagcaaggacagcacctacagcctcagcagcaccctgacgctgagcaaagcagactacgagaaacacaaagtctacgcctgcgaagtcacccatcagggcctgagctcgcccgtcacaaagagcttcaacaggggagagtgttag

SEQ ID NO: 15 - protein, 8 aa, Artificial Sequence
  VH-CDR1
GYSFTGYY

SEQ ID NO: 16 - protein, 8 aa, Artificial Sequence
  VH-CDR2
INPYNGAT

SEQ ID NO: 17 - protein, 10 aa, Artificial Sequence
  VH-CDR3
ARFHYGAPDY

SEQ ID NO: 18 - protein, 6 aa, Artificial Sequence
  VL-CDR1
QDINTY

SEQ ID NO: 19 - protein, 3 aa, Artificial Sequence
  VL-CDR2
RAN

SEQ ID NO: 20 - protein, 9 aa, Artificial Sequence
  VL-CDR3
LQYDEFPLT

SEQ ID NO: 21 - protein, 8 aa, Artificial Sequence
  137-1VH-CDR1
GYTFTGYY

SEQ ID NO: 22 - protein, 10 aa, Artificial Sequence
  137-4VH-CDR3
ARFHYGAVDY

SEQ ID NO: 23 - protein, 10 aa, Artificial Sequence
  137-5VH-CDR3
ARFHYGAADY

SEQ ID NO: 24 - protein, 10 aa, Artificial Sequence
  137-6VH-CDR3
ARFHYGAPEY

SEQ ID NO: 25 - protein, 10 aa, Artificial Sequence
  137-7VH-CDR3
ARFHYGAPNY

SEQ ID NO: 26 - protein, 10 aa, Artificial Sequence
  137-8VH-CDR3
ARFHYGAPDF

SEQ ID NO: 27 - protein, 10 aa, Artificial Sequence
  137-9VH-CDR3
ARFHYGAPDL

SEQ ID NO: 28 - protein, 9 aa, Artificial Sequence
  137-4VL-CDR3
LQYEEFPLT

SEQ ID NO: 29 - protein, 9 aa, Artificial Sequence
  137-5VL-CDR3
LQYNEFPLT

SEQ ID NO: 30 - protein, 9 aa, Artificial Sequence
  137-6VL-CDR3
LQYAEFPLT

SEQ ID NO: 31 - protein, 9 aa, Artificial Sequence
  137-7VL-CDR3
LQYDDFPLT

SEQ ID NO: 32 - protein, 9 aa, Artificial Sequence
  137-8VL-CDR3
LQYDQFPLT

SEQ ID NO: 33 - protein, 9 aa, Artificial Sequence
  137-9VL-CDR3
LQYDAFPLT

SEQ ID NO: 34 - protein, 117 aa, Artificial Sequence
  137-4 VH
QVQLVQSGAEVKKPGSSVKVSCKASGYSFTGYYIHWVRQAPGQGLEWMGRINPYNGATTYNQNFKDRVTITVDKSTSTAYMELSSLRSEDTAVYYCARFHYGAVDYWGQGTLVTVSS

SEQ ID NO: 35 - protein, 117 aa, Artificial Sequence
  137-5 VH
QVQLVQSGAEVKKPGSSVKVSCKASGYSFTGYYIHWVRQAPGQGLEWMGRINPYNGATTYNQNFKDRVTITVDKSTSTAYMELSSLRSEDTAVYYCARFHYGAADYWGQGTLVTVSS

SEQ ID NO: 36 - protein, 117 aa, Artificial Sequence
  137-6 VH
QVQLVQSGAEVKKPGSSVKVSCKASGYSFTGYYIHWVRQAPGQGLEWMGRINPYNGATTYNQNFKDRVTITVDKSTSTAYMELSSLRSEDTAVYYCARFHYGAPEYWGQGTLVTVSS

SEQ ID NO: 37 - protein, 117 aa, Artificial Sequence
  137-7 VH
QVQLVQSGAEVKKPGSSVKVSCKASGYSFTGYYIHWVRQAPGQGLEWMGRINPYNGATTYNQNFKDRVTITVDKSTSTAYMELSSLRSEDTAVYYCARFHYGAPNYWGQGTLVTVSS

SEQ ID NO: 38 - protein, 117 aa, Artificial Sequence
  137-8 VH
QVQLVQSGAEVKKPGSSVKVSCKASGYSFTGYYIHWVRQAPGQGLEWMGRINPYNGATTYNQNFKDRVTITVDKSTSTAYMELSSLRSEDTAVYYCARFHYGAPDFWGQGTLVTVSS

SEQ ID NO: 39 - protein, 117 aa, Artificial Sequence
  137-9 VH
QVQLVQSGAEVKKPGSSVKVSCKASGYSFTGYYIHWVRQAPGQGLEWMGRINPYNGATTYNQNFKDRVTITVDKSTSTAYMELSSLRSEDTAVYYCARFHYGAPDLWGQGTLVTVSS

SEQ ID NO: 40 - protein, 108 aa, Artificial Sequence
  137-4 VL
DIQMTQSPSSLSASVGDRVTITCKASQDINTYLTWYQQKPGKAPKTLIYRANILVDGVPSRFSGSGSGTDFTLTISSLQPEDFATYYCLQYEEFPLTFGGGTKVEIKR

SEQ ID NO: 41 - protein, 108 aa, Artificial Sequence
  137-5 VL
DIQMTQSPSSLSASVGDRVTITCKASQDINTYLTWYQQKPGKAPKTLIYRANILVDGVPSRFSGSGSGTDFTLTISSLQPEDFATYYCLQYNEFPLTFGGGTKVEIKR

SEQ ID NO: 42 - protein, 108 aa, Artificial Sequence
  137-6 VL
DIQMTQSPSSLSASVGDRVTITCKASQDINTYLTWYQQKPGKAPKTLIYRANILVDGVPSRFSGSGSGTDFTLTISSLQPEDFATYYCLQYAEFPLTFGGGTKVEIKR

SEQ ID NO: 43 - protein, 108 aa, Artificial Sequence
  137-7 VL
DIQMTQSPSSLSASVGDRVTITCKASQDINTYLTWYQQKPGKAPKTLIYRANILVDGVPSRFSGSGSGTDFTLTISSLQPEDFATYYCLQYDDFPLTFGGGTKVEIKR

SEQ ID NO: 44 - protein, 108 aa, Artificial Sequence
  137-8 VL
DIQMTQSPSSLSASVGDRVTITCKASQDINTYLTWYQQKPGKAPKTLIYRANILVDGVPSRFSGSGSGTDFTLTISSLQPEDFATYYCLQYDQFPLTFGGGTKVEIKR

SEQ ID NO: 45 - protein, 108 aa, Artificial Sequence
  137-9 VL
DIQMTQSPSSLSASVGDRVTITCKASQDINTYLTWYQQKPGKAPKTLIYRANILVDGVPSRFSGSGSGTDFTLTISSLQPEDFATYYCLQYDAFPLTFGGGTKVEIKR

SEQ ID NO: 46 - protein, 330 aa, Artificial Sequence [sequence omitted]

SEQ ID NO: 47 - protein, 106 aa, Artificial Sequence; identical to SEQ ID NO: 4
  kappa chain constant region